European Patent Application EP 4 491 194 A1, published January 15, 2025. Title: 두경부암 치료를 위한 삼중 복합약물 투여요법. Applicant: Genexine, Inc. The sequence listing filed with the application follows.

SEQUENCE LISTING (55 sequences)

SEQ ID NO: 1 - DNA, 477 bp, synthetic construct
  source 1..477: mol_type = other DNA
atgcaccaaaagagaactgcaatgtttcaggacccacaggagcgacccagaaagttaccacatttatgcacagagctgcaaacaactatacatgatataatattagaatgtgtgtactgcaagcaacagttactgcgacgtgaggtatatgactttgcttttcgggatttatgcatagtatatagagatgggaatccatatgcagtgtgtgataaatgtttaaagttttattctaaaattagtgagtatagatattattgttatagtgtgtatggaacaacattagaacagcaatacaacaaaccgttgtgtgatttgttaattaggtgtattaactgtcaaaagccactgtgtcctgaagaaaagcaaagacatctggacaaaaagcaaagattccataatataaggggtcggtggaccggtcgatgtatgtcttgttgcagatcatcaagaacacgtagagaaacccagctgtaa

SEQ ID NO: 2 - protein, 158 aa, synthetic construct
MHQKRTAMFQDPQERPRKLPHLCTELQTTIHDIILECVYCKQQLLRREVYDFAFRDLCIVYRDGNPYAVCDKCLKFYSKISEYRYYCYSVYGTTLEQQYNKPLCDLLIRCINCQKPLCPEEKQRHLDKKQRFHNIRGRWTGRCMSCCRSSRTRRETQL

SEQ ID NO: 3 - DNA, 477 bp, synthetic construct
  source 1..477: mol_type = other DNA
atggcgcgctttgaggatccaacacggcgaccctacaagctacctgatctgtgcacggaactgaacacttcactgcaagacatagaaataacctgtgtatattgcaagacagtattggaacttacagaggtatttgaatttgcattcaaagatttatttgtagtgtatagagacagtataccgcatgctgcatgccataaatgtatagatttctattctagaattagagaattaagatattattcagactctgtgtatggagacacattagaaaaactaactaacactgggttatacaatttattaataaggtgcctgcggtgccagaaaccgttgaatccagcagaaaaacttagacaccttaatgaaaaacgacgattccacaaaatagctgggcactatagaggccagtgccattcgtgctgcaaccgagcacgacaggagagactccaacgacgcagagaaacacaagtataa

SEQ ID NO: 4 - protein, 158 aa, synthetic construct
MARFEDPTRRPYKLPDLCTELNTSLQDIEITCVYCKTVLELTEVFEFAFKDLFVVYRDSIPHAACHKCIDFYSRIRELRYYSDSVYGDTLEKLTNTGLYNLLIRCLRCQKPLNPAEKLRHLNEKRRFHKIAGHYRGQCHSCCNRARQERLQRRRETQV

SEQ ID NO: 5 - DNA, 297 bp, synthetic construct
  source 1..297: mol_type = other DNA
atgcatggagatacacctacattgcatgaatatatgttagatttgcaaccagagacaactgatctctactgttatgagcaattaaatgacagctcagaggaggaggatgaaatagatggtccagctggacaagcagaaccggacagagcccattacaatattgtaaccttttgttgcaagtgtgactctacgcttcggttgtgcgtacaaagcacacacgtagacattcgtactttggaagacctgttaatgggcacactaggaattgtgtgccccatctgttctcagaaaccataa

SEQ ID NO: 6 - protein, 98 aa, synthetic construct
MHGDTPTLHEYMLDLQPETTDLYCYEQLNDSSEEEDEIDGPAGQAEPDRAHYNIVTFCCKCDSTLRLCVQSTHVDIRTLEDLLMGTLGIVCPICSQKP

SEQ ID NO: 7 - DNA, 318 bp, synthetic construct
  source 1..318: mol_type = other DNA
atgtatggacctaaggcaacattgcaagacattgtattgcatttagagcctcaaaatgaaattccggttgaccttctatgtcacgagcaattaagcgactcagaggaagaaaacgatgaaatagatggagttaatcatcaacatttaccagcccgacgagccgaaccacaacgtcacacaatgttgtgtatgtgttgtaagtgtgaagccagaattgagctagtagtagaaagctcagcagacgaccttcgagcattccagcagctgtttctgagcaccctgtcctttgtgtgtccgtggtgtgcatcccagcagtaa

SEQ ID NO: 8 - protein, 105 aa, synthetic construct
MYGPKATLQDIVLHLEPQNEIPVDLLCHEQLSDSEEENDEIDGVNHQHLPARRAEPQRHTMLCMCCKCEARIELVVESSADDLRAFQQLFLSTLSFVCPWCASQQ

SEQ ID NO: 9 - DNA, 1737 bp, synthetic construct
  source 1..1737: mol_type = other DNA
atgcaccagaagagaaccgccatgttccaggaccctcaggagagacctaggaagctgcctcacctgtgtacagagctccagacaaccatccacgacatcatcctggagtgcgtgtactgtaagcagcagctgctgagaagagaggtgtacgacttcgccttcagagacctgtgcatcgtgtacagagacggcaacccttacgccgtgtgcgataagtgtctgaagttctattccaaaatctccgaatataggtacatgcacggcgacacccctaccctgcacgagtacatgctggacctccagcctgagaccacagacctgtactgctacgagcagctgaacgacagctctgaggaagaggacgagattgacggacctgctggccaggccgagcctgacagagcccactacaatatcgtgacattctgttgcaaatgcgactccacactggacaagtgcctgaagttctacagcaagatctctgagtacagatactactgctactctgtgtacggcaccacactggagcagcagtacaacaagcctctgtgcgacctcctgatccgctgcatcaactgccagaagcctctgtgccctgaggagaagcagagacacctggacaagaagcagcggttccacaacatcagaggcagatggaccggcaggtgcatgtcctgctgtagatcctccagaaccagacgggagacccagctgcactacaacatcgtgaccttctgctgcaagtgcgactctaccctgagactgtgcgtgcagtctacccacgtggacatcagaaccctggaggacctgctgatgggcaccctgggcatcgtgtgccctatctgctctcagaagcctatggccaggttcgaggaccctaccagaagaccctacaagctgcctgacctgtgcaccgagctgaacacctctctgcaagacatcgagatcacctgcgtgtactgcaagaccgtgctggagctgaccgaggtgttcgagttcgccttcaaggacctgttcgtggtgtacagagacagcatccctcacgctgcctgccacaagtgcatcgacttctattccaggatcagggagctgcgctattactccgactctgtgatgtacggccccaaggccaccctccaggacatcgtgctgcacctggagcctcagaacgagatccccgtggacctgctgtgccacgagcagctgtctgactctgaagaggagaacgacgagatcgacggcgtgaaccaccagcacctgcctgccaggagagctgaaccccagcggcataccatgctgtgtatgtgcttctactctaggatcagagagctgaggtactactctgactctgtgtacggcgacaccctggagaagctgaccaacaccggcctgtacaacctgctgatccggtgcctgaggtgccagaagcctctgaaccctgccgagaagctgagacacctgaacgagaagagaagattccacaagatcgctggccactacagaggccagtgccactcttgctgcaacagagccagacaggagagactccagcggagaagggagacccaggtggccagaagagccgagcctcagagacacaccatgctgtgcatgtgctgcaagtgcgaggccagaatcgagctggtggtggagagctctgccgacgacctgagagccttccagcagctgttcctgtctaccctgagcttcgtgtgcccttggtgcgcctctcagcag

SEQ ID NO: 10 - protein, 579 aa, synthetic construct
MHQKRTAMFQDPQERPRKLPHLCTELQTTIHDIILECVYCKQQLLRREVYDFAFRDLCIVYRDGNPYAVCDKCLKFYSKISEYRYMHGDTPTLHEYMLDLQPETTDLYCYEQLNDSSEEEDEIDGPAGQAEPDRAHYNIVTFCCKCDSTLDKCLKFYSKISEYRYYCYSVYGTTLEQQYNKPLCDLLIRCINCQKPLCPEEKQRHLDKKQRFHNIRGRWTGRCMSCCRSSRTRRETQLHYNIVTFCCKCDSTLRLCVQSTHVDIRTLEDLLMGTLGIVCPICSQKPMARFEDPTRRPYKLPDLCTELNTSLQDIEITCVYCKTVLELTEVFEFAFKDLFVVYRDSIPHAACHKCIDFYSRIRELRYYSDSVMYGPKATLQDIVLHLEPQNEIPVDLLCHEQLSDSEEENDEIDGVNHQHLPARRAEPQRHTMLCMCFYSRIRELRYYSDSVYGDTLEKLTNTGLYNLLIRCLRCQKPLNPAEKLRHLNEKRRFHKIAGHYRGQCHSCCNRARQERLQRRRETQVARRAEPQRHTMLCMCCKCEARIELVVESSADDLRAFQQLFLSTLSFVCPWCASQQ

SEQ ID NO: 11 - DNA, 489 bp, synthetic construct
  source 1..489: mol_type = other DNA
atcacccaggactgctccttccaacacagccccatctcctccgacttcgctgtcaaaatccgtgagctgtctgactacctgcttcaagattacccagtcaccgtggcctccaacctgcaggacgaggagctctgcgggggcctctggcggctggtcctggcacagcgctggatggagcggctcaagactgtcgctgggtccaagatgcaaggcttgctggagcgcgtgaacacggagatacactttgtcaccaaatgtgcctttcagcccccccccagctgtcttcgcttcgtccagaccaacatctcccgcctcctgcaggagacctccgagcagctggtggcgctgaagccctggatcactcgccagaacttctcccggtgcctggagctgcagtgtcagcccgactcctcaaccctgccacccccatggagtccccggcccctggaggccacagccccgacagccccgggcggcggcagcggcgat

SEQ ID NO: 12 - protein, 163 aa, synthetic construct
ITQDCSFQHSPISSDFAVKIRELSDYLLQDYPVTVASNLQDEELCGGLWRLVLAQRWMERLKTVAGSKMQGLLERVNTEIHFVTKCAFQPPPSCLRFVQTNISRLLQETSEQLVALKPWITRQNFSRCLELQCQPDSSTLPPPWSPRPLEATAPTAPGGGSGD

SEQ ID NO: 13 - DNA, 69 bp, synthetic construct
  source 1..69: mol_type = other DNA
atggatgctatgaaacggggcctgtgctgcgtgctgctcctgtgcggcgctgtgtttgtgagccctagc

SEQ ID NO: 14 - protein, 23 aa, synthetic construct
MDAMKRGLCCVLLLCGAVFVSPS

SEQ ID NO: 15 - DNA, 6085 bp, synthetic construct
  source 1..6085: mol_type = other DNA
acgcgttgacattgattattgactagttattaatagtaatcaattacggggtcattagttcatagcccatatatggagttccgcgttacataacttacggtaaatggcccgcctggctgaccgcccaacgacccccgcccattgacgtcaataatgacgtatgttcccatagtaacgccaatagggactttccattgacgtcaatgggtggagtatttacggtaaactgcccacttggcagtacatcaagtgtatcatatgccaagtacgccccctattgacgtcaatgacggtaaatggcccgcctggcattatgcccagtacatgaccttatgggactttcctacttggcagtacatctacgtattagtcatcgctattaccatggtgatgcggttttggcagtacatcaatgggcgtggatagcggtttgactcacggggatttccaagtctccaccccattgacgtcaatgggagtttgttttggcaccaaaatcaacgggactttccaaaatgtcgtaacaactccgccccattgacgcaaatgggcggtaggcgtgtacggtgggaggtctatataagcagagctctctggctaactagagaacccactgcttactggcttatcgaaattaatacgactcactatagggagacccaagctggctagcgtgagtttggggacccttgattgttctttctttttcgctattgtaaaattcatgttatatggagggggcaaagttttcagggtgttgtttagaacgggaagatgtcccttgtatcaccatggaccctcatgataattttgtttctttcactttctactctgttgacaaccattgtctcctcttattttcttttcattttctgtaactttttcgttaaactttagcttgcatttgtaacgaatttttaaattcacttttgtttatttgtcagattgtaagtactttctctaatcacttttttttcaaggcaatcagggtatattatattgtacttcagcacagttttagagaacaattgttataattaaatgataaggtagaatatttctgcatataaattctggctggcgtggaaatattcttattggtagaaacaactacatcctggtcatcatcctgcctttctctttatggttacaatgatatacactgtttgagatgaggataaaatactctgagtccaaaccgggcccctctgctaaccatgttcatgccttcttctttttcctacagctcctgggcaacgtgctggttattgtgctgtctcatcattttggcaaagaattgtaatacgactcactatagggcgaattgaagcttggtaccgccaccatggatgctatgaaacggggcctgtgctgcgtgctgctcctgtgcggcgctgtgtttgtgagccctagcatcacccaggactgctccttccaacacagccccatctcctccgacttcgctgtcaaaatccgtgagctgtctgactacctgcttcaagattacccagtcaccgtggcctccaacctgcaggacgaggagctctgcgggggcctctggcggctggtcctggcacagcgctggatggagcggctcaagactgtcgctgggtccaagatgcaaggcttgctggagcgcgtgaacacggagatacactttgtcaccaaatgtgcctttcagcccccccccagctgtcttcgcttcgtccagaccaacatctcccgcctcctgcaggagacctccgagcagctggtggcgctgaagccctggatcactcgccagaacttctcccggtgcctggagctgcagtgtcagcccgactcctcaaccctgccacccccatggagtccccggcccctggaggccacagccccgacagccccgggcggcggcagcggcgatgctagcatgcaccagaagagaaccgccatgttccaggaccctcaggagagacctaggaagctgcctcacctgtgtacagagctccagacaaccatccacgacatcatcctggagtgcgtgtactgtaagcagcagctgctgagaagagaggtgtacgacttcgccttcagagacctgtgcatcgtgtacagagacggcaacccttacgccgtgtgcgataagtgtctgaagttctattccaaaatctccgaatataggtacatgcacggcgacacccctaccctgcacgagtacatgctggacctccagcctgagaccacagacctgtactgctacgagcagctgaacgacagctctgaggaagaggacgagattgacggacctgctggccaggccgagcctgacagagcccactacaatatcgtgacattctgttgcaaatgcgactccacactggacaagtgcctgaagttctacagcaagatctctgagtacagatactactgctactctgtgtacggcaccacactggagcagcagtacaacaagcctctgtgcgacctcctgatccgctgcatcaactgccagaagcctctgtgccctgaggagaagcagagacacctggacaagaagcagcggttccacaacatcagaggcagatggaccggcaggtgcatgtcctgctgtagatcctccagaaccagacgggagacccagctgcactacaacatcgtgaccttctgctgcaagtgcgactctaccctgagactgtgcgtgcagtctacccacgtggacatcagaaccctggaggacctgctgatgggcaccctgggcatcgtgtgccctatctgctctcagaagcctatggccaggttcgaggaccctaccagaagaccctacaagctgcctgacctgtgcaccgagctgaacacctctctgcaagacatcgagatcacctgcgtgtactgcaagaccgtgctggagctgaccgaggtgttcgagttcgccttcaaggacctgttcgtggtgtacagagacagcatccctcacgctgcctgccacaagtgcatcgacttctattccaggatcagggagctgcgctattactccgactctgtgatgtacggccccaaggccaccctccaggacatcgtgctgcacctggagcctcagaacgagatccccgtggacctgctgtgccacgagcagctgtctgactctgaagaggagaacgacgagatcgacggcgtgaaccaccagcacctgcctgccaggagagctgaaccccagcggcataccatgctgtgtatgtgcttctactctaggatcagagagctgaggtactactctgactctgtgtacggcgacaccctggagaagctgaccaacaccggcctgtacaacctgctgatccggtgcctgaggtgccagaagcctctgaaccctgccgagaagctgagacacctgaacgagaagagaagattccacaagatcgctggccactacagaggccagtgccactcttgctgcaacagagccagacaggagagactccagcggagaagggagacccaggtggccagaagagccgagcctcagagacacaccatgctgtgcatgtgctgcaagtgcgaggccagaatcgagctggtggtggagagctctgccgacgacctgagagccttccagcagctgttcctgtctaccctgagcttcgtgtgcccttggtgcgcctctcagcagtaatctagagtcggggcggccggccgcttcgagcagacatgataagatacattgatgagtttggacaaaccacaactagaatgcagtgaaaaaaatgctttatttgtgaaatttgtgatgctattgctttatttgtaaccattataagctgcaataaacaagttaacaacaacaattgcattcattttatgtttcaggttcagggggaggtgtgggaggttttttaaagcaagtaaaacctctacaaatgtggtaaaatcgataaggatctgaacgatggagcggagaatgggcggaactgggcggagttaggggcgggatgggcggagttaggggcgggactatggttgctgactaattgagatgcatgctttgcatacttctgcctgctggggagcctggggactttccacacctggttgctgactaattgagatgcatgctttgcatacttctgcctgctggggagcctggggactttccacaccctaactgacacacattccacagcggatccgtcgacttcagaagaactcgtcaagaaggcgatagaaggcgatgcgccgcgaatcgggagcggcgataccgtagagcacgaggaagcggtcagcccattcgccgccaagctcttcagcaatatcacgggtagccaacgctatgtcctgatagcggtccgccacacccagccggccacagtcgatgaatccagaaaagcggccattttccaccatgatattcggcaagcaggcatcgccatgggtcacgacgagatcctcgccgtcgggcatgctcgccttgagcctggcgaacagttcggctggcgcgagcccctgatgctcttcgtccagatcatcctgatcgacaagaccggcttccatccgagtacgtgctcgctcgatgcgatgtttcgcttggtggtcgaatgggcaggtagccggatcaagcgtatgcagccgccgcattgcatcagccatgatggatactttctcggcaggagcaaggtgagatgacaggagatcctgccccggcacttcgcccaatagcagccagtcccttcccgcttcagtgacaacgtcgagcacagctgcgcaaggaacgcccgtcgtggccagccacgatagccgcgctgcctcgtcttgcagttcattcagggcaccggacaggtcggtcttgacaaaaagaaccgggcgcccctgcgctgacagccggaacacggcggcatcagagcagccgattgtctgttgtgcccagtcatagccgaatagcctctccacccaagcggccggagaacctgcgtgcaatccatcttgttcaatcatgcgaaacgatcctcatcctgtctcttgatcagatcttgatcccctgcgccatcagatccttggcggcaagaaagccatccagtttactttgcagggcttcccaaccttaccagagggcgccccagctggcaattccggttcgcttgctgtccataaaaccgcccagtctagctatcgccatgtaagcccactgcaagctacctgctttctctttgcgcttgcgttttcccttgtccagatagcccagtagctgacattcatccggggtcagcaccgtttctgcggactggctttctacgtgaaaaggatctaggtgaagatcctttttgataatctcatgaccaaaatcccttaacgtgagttttcgttccactgagcgtcagaccccgtagaaaagatcaaaggatcttcttgagatcctttttttctgcgcgtaatctgctgcttgcaaacaaaaaaaccaccgctaccagcggtggtttgtttgccggatcaagagctaccaactctttttccgaaggtaactggcttcagcagagcgcagataccaaatactgttcttctagtgtagccgtagttaggccaccacttcaagaactctgtagcaccgcctacatacctcgctctgctaatcctgttaccagtggctgctgccagtggcgataagtcgtgtcttaccgggttggactcaagacgatagttaccggataaggcgcagcggtcgggctgaacggggggttcgtgcacacagcccagcttggagcgaacgacctacaccgaactgagatacctacagcgtgagctatgagaaagcgccacgcttcccgaagggagaaaggcggacaggtatccggtaagcggcagggtcggaacaggagagcgcacgagggagcttccagggggaaacgcccggtatctttatagtcctgtcgggtttcgccacctctgacttgagcgtcgatttttgtgatgctcgtcaggggggcggagcctatggaaaaacgccagcaacgcggcctttttacggttcctggccttttgctggccttttgctcacatgttcgggcccaatcgacccgggcgacggccagtgaattgtaccgatgtacgggccagatat

SEQ ID NO: 16 - protein, 152 aa, Homo sapiens
DCDIEGKDGKQYESVLMVSIDQLLDSMKEIGSNCLNNEFNFFKRHICDANKEGMFLFRAARKLRQFLKMNSTGDFDLHLLKVSEGTTILLNCTGQVKGRKPAALGEAQPTKSLEENKSLKEQKKLNDLCFLKRLLQEIKTCWNKILMGTKEH

SEQ ID NO: 17 - protein, 154 aa, Rattus norvegicus
MFHVSFRYIFGIPPLILVLLPVTSSDCHIKDKDGKAFGSVLMISINQLDKMTGTDSDCPNNEPNFFKKHLCDDTKEAAFLNRAARKLRQFLKMNISEEFNDHLLRVSDGTQTLVNCTSKEEKTIKEQKKNDPCFLKRLLREIKTCWNKILKGSI

SEQ ID NO: 18 - protein, 154 aa, Mus musculus
MFHVSFRYIFGIPPLILVLLPVTSSECHIKDKEGKAYESVLMISIDELDKMTGTDSNCPNNEPNFFRKHVCDDTKEAAFLNRAARKLKQFLKMNISEEFNVHLLTVSQGTQTLVNCTSKEEKNVKEQKKNDACFLKRLLREIKTCWNKILKGSI

SEQ ID NO: 19 - protein, 177 aa, Chlorocebus sabaeus
MFHVSFRYIFGLPPLILVLLPVASSDCDIEGKDGKQYESVLMVSIDQLLDSMKEIGSNCLNNEFNFFKRHLCDDNKEGMFLFRAARKLKQFLKMNSTGDFDLHLLKVSEGTTILLNCTGKVKGRKPAALGEPQPTKSLEENKSLKEQKKLNDSCFLKRLLQKIKTCWNKILMGTKEH

SEQ ID NO: 20 - protein, 176 aa, Bos taurus
MFHVSFRYIFGIPPLILVLLPVASSDCDISGKDGGAYQNVLMVNIDDLDNMINFDSNCLNNEPNFFKKHSCDDNKEASFLNRASRKLRQFLKMNISDDFKLHLSTVSQGTLTLLNCTSKGKGRKPPSLSEAQPTKNLEENKSSKEQKKQNDLCFLKILLQKIKTCWNKILRGIKEH

SEQ ID NO: 21 - protein, 176 aa, Ovis aries
MFHVSFRYIFGIPPLILVLLPVASSDCDFSGKDGGAYQNVLMVSIDDLDNMINFDSNCLNNEPNFFKKHSCDDNKEASFLNRAARKLKQFLKMNISDDFKLHLSTVSQGTLTLLNCTSKGKGRKPPSLGEAQPTKNLEENKSLKEQRKQNDLCFLKILLQKIKTCWNKILRGITEH

SEQ ID NO: 22 - protein, 384 aa, Homo sapiens
APTKAPDVFPIISGCRHPKDNSPVVLACLITGYHPTSVTVTWYMGTQSQPQRTFPEIQRRDSYYMTSSQLSTPLQQWRQGEYKCVVQHTASKSKKEIFRWPESPKAQASSVPTAQPQAEGSLAKATTAPATTRNTGRGGEEKKKEKEKEEQEERETKTPECPSHTQPLGVYLLTPAVQDLWLRDKATFTCFVVGSDLKDAHLTWEVAGKVPTGGVEEGLLERHSNGSQSQHSRLTLPRSLWNAGTSVTCTLNHPSLPPQRLMALREPAAQAPVKLSLNLLASSDPPEAASWLLCEVSGFSPPNILLMWLEDQREVNTSGFAPARPPPQPGSTTFWAWSVLRVPAPPSPQPATYTCVVSHEDSRTLLNASRSLEVSYVTDHGPMK

SEQ ID NO: 23 - protein, 327 aa, Homo sapiens
ASTKGPSVFPLAPCSRSTSESTAALGCLVKDYFPEPVTVSWNSGALTSGVHTFPAVLQSSGLYSLSSVVTVPSSSLGTKTYTCNVDHKPSNTKVDKRVESKYGPPCPSCPAPEFLGGPSVFLFPPKPKDTLMISRTPEVTCVVVDVSQEDPEVQFNWYVDGVEVHNAKTKPREEQFNSTYRVVSVLTVLHQDWLNGKEYKCKVSNKGLPSSIEKTISKAKGQPREPQVYTLPPSQEEMTKNQVSLTCLVKGFYPSDIAVEWESNGQPENNYKTTPPVLDSDGSFFLYSRLTVDKSRWQEGNVFSCSVMHEALHNHYTQKSLSLSLGK

SEQ ID NO: 24 - protein, 245 aa, synthetic construct
RNTGRGGEEKKKEKEKEEQEERETKTPECPSHTQPLGVFLFPPKPKDTLMISRTPEVTCVVVDVSQEDPEVQFNWYVDGVEVHNAKTKPREEQFNSTYRVVSVLTVLHQDWLNGKEYKCKVSNKGLPSSIEKTISKAKGQPREPQVYTLPPSQEEMTKNQVSLTCLVKGFYPSDIAVEWESNGQPENNYKTTPPVLDSDGSFFLYSRLTVDKSRWQEGNVFSCSVMHEALHNHYTQKSLSLSLGK

SEQ ID NO: 25 - protein, 245 aa, synthetic construct
RNTGRGGEEKKGGKEKEEQEERETKTPECPSHTQPLGVFLFPPKPKDTLMISRTPEVTCVVVDVSQEDPEVQFNWYVDGVEVHNAKTKPREEQFNSTYRVVSVLTVLHQDWLNGKEYKCKVSNKGLPSSIEKTISKAKGQPREPQVYTLPPSQEEMTKNQVSLTCLVKGFYPSDIAVEWESNGQPENNYKTTPPVLDSDGSFFLYSRLTVDKSRWQEGNVFSCSVMHEALHNHYTQKSLSLSLGK

SEQ ID NO: 26 - protein, 245 aa, synthetic construct
RNTGRGGEEKKGSKEKEEQEERETKTPECPSHTQPLGVFLFPPKPKDTLMISRTPEVTCVVVDVSQEDPEVQFNWYVDGVEVHNAKTKPREEQFNSTYRVVSVLTVLHQDWLNGKEYKCKVSNKGLPSSIEKTISKAKGQPREPQVYTLPPSQEEMTKNQVSLTCLVKGFYPSDIAVEWESNGQPENNYKTTPPVLDSDGSFFLYSRLTVDKSRWQEGNVFSCSVMHEALHNHYTQKSLSLSLGK

SEQ ID NO: 27 - protein, 245 aa, synthetic construct
RNTGRGGEEKKSGKEKEEQEERETKTPECPSHTQPLGVFLFPPKPKDTLMISRTPEVTCVVVDVSQEDPEVQFNWYVDGVEVHNAKTKPREEQFNSTYRVVSVLTVLHQDWLNGKEYKCKVSNKGLPSSIEKTISKAKGQPREPQVYTLPPSQEEMTKNQVSLTCLVKGFYPSDIAVEWESNGQPENNYKTTPPVLDSDGSFFLYSRLTVDKSRWQEGNVFSCSVMHEALHNHYTQKSLSLSLGK

SEQ ID NO: 28 - protein, 245 aa, synthetic construct
RNTGRGGEEKKSSKEKEEQEERETKTPECPSHTQPLGVFLFPPKPKDTLMISRTPEVTCVVVDVSQEDPEVQFNWYVDGVEVHNAKTKPREEQFNSTYRVVSVLTVLHQDWLNGKEYKCKVSNKGLPSSIEKTISKAKGQPREPQVYTLPPSQEEMTKNQVSLTCLVKGFYPSDIAVEWESNGQPENNYKTTPPVLDSDGSFFLYSRLTVDKSRWQEGNVFSCSVMHEALHNHYTQKSLSLSLGK

SEQ ID NO: 29 - protein, 243 aa, synthetic construct
ASAEPRGPTIKPCPPCKCPAPNLEGGPSVFIFPPKIKDVLMISLSPIVTCVVVDVSEDDPDVQISWFVNNVEVHTAQTQTHREDYNSTLRVVSALPIQHQDWMSGKAFACAVNNKDLPAPIERTISKPKGSVRAPQVYVLPPPEEEMTKKQVTLTCMVTDFMPEDIYVEWTNNGKTELNYKNTEPVLDSDGSYFMYSKLRVEKKNWVERNSYSCSVVHEGLHNHHTTKSFSRTPGKGGGNSGS

SEQ ID NO: 30 - protein, 153 aa, synthetic construct
MDCDIEGKDGKQYESVLMVSIDQLLDSMKEIGSNCLNNEFNFFKRHICDANKEGMFLFRAARKLRQFLKMNSTGDFDLHLLKVSEGTTILLNCTGQVKGRKPAALGEAQPTKSLEENKSLKEQKKLNDLCFLKRLLQEIKTCWNKILMGTKEH

SEQ ID NO: 31 - protein, 154 aa, synthetic construct
MMDCDIEGKDGKQYESVLMVSIDQLLDSMKEIGSNCLNNEFNFFKRHICDANKEGMFLFRAARKLRQFLKMNSTGDFDLHLLKVSEGTTILLNCTGQVKGRKPAALGEAQPTKSLEENKSLKEQKKLNDLCFLKRLLQEIKTCWNKILMGTKEH

SEQ ID NO: 32 - protein, 155 aa, synthetic construct
MMMDCDIEGKDGKQYESVLMVSIDQLLDSMKEIGSNCLNNEFNFFKRHICDANKEGMFLFRAARKLRQFLKMNSTGDFDLHLLKVSEGTTILLNCTGQVKGRKPAALGEAQPTKSLEENKSLKEQKKLNDLCFLKRLLQEIKTCWNKILMGTKEH

SEQ ID NO: 33 - protein, 155 aa, synthetic construct
MGMDCDIEGKDGKQYESVLMVSIDQLLDSMKEIGSNCLNNEFNFFKRHICDANKEGMFLFRAARKLRQFLKMNSTGDFDLHLLKVSEGTTILLNCTGQVKGRKPAALGEAQPTKSLEENKSLKEQKKLNDLCFLKRLLQEIKTCWNKILMGTKEH

SEQ ID NO: 34 - protein, 155 aa, synthetic construct
DDDDCDIEGKDGKQYESVLMVSIDQLLDSMKEIGSNCLNNEFNFFKRHICDANKEGMFLFRAARKLRQFLKMNSTGDFDLHLLKVSEGTTILLNCTGQVKGRKPAALGEAQPTKSLEENKSLKEQKKLNDLCFLKRLLQEIKTCWNKILMGTKEH

SEQ ID NO: 35 - protein, 156 aa, synthetic construct
MMMMDCDIEGKDGKQYESVLMVSIDQLLDSMKEIGSNCLNNEFNFFKRHICDANKEGMFLFRAARKLRQFLKMNSTGDFDLHLLKVSEGTTILLNCTGQVKGRKPAALGEAQPTKSLEENKSLKEQKKLNDLCFLKRLLQEIKTCWNKILMGTKEH

SEQ ID NO: 36 - protein, 398 aa, synthetic construct
MDCDIEGKDGKQYESVLMVSIDQLLDSMKEIGSNCLNNEFNFFKRHICDANKEGMFLFRAARKLRQFLKMNSTGDFDLHLLKVSEGTTILLNCTGQVKGRKPAALGEAQPTKSLEENKSLKEQKKLNDLCFLKRLLQEIKTCWNKILMGTKEHRNTGRGGEEKKKEKEKEEQEERETKTPECPSHTQPLGVFLFPPKPKDTLMISRTPEVTCVVVDVSQEDPEVQFNWYVDGVEVHNAKTKPREEQFNSTYRVVSVLTVLHQDWLNGKEYKCKVSNKGLPSSIEKTISKAKGQPREPQVYTLPPSQEEMTKNQVSLTCLVKGFYPSDIAVEWESNGQPENNYKTTPPVLDSDGSFFLYSRLTVDKSRWQEGNVFSCSVMHEALHNHYTQKSLSLSLGK

SEQ ID NO: 37 - protein, 399 aa, synthetic construct
MMDCDIEGKDGKQYESVLMVSIDQLLDSMKEIGSNCLNNEFNFFKRHICDANKEGMFLFRAARKLRQFLKMNSTGDFDLHLLKVSEGTTILLNCTGQVKGRKPAALGEAQPTKSLEENKSLKEQKKLNDLCFLKRLLQEIKTCWNKILMGTKEHRNTGRGGEEKKKEKEKEEQEERETKTPECPSHTQPLGVFLFPPKPKDTLMISRTPEVTCVVVDVSQEDPEVQFNWYVDGVEVHNAKTKPREEQFNSTYRVVSVLTVLHQDWLNGKEYKCKVSNKGLPSSIEKTISKAKGQPREPQVYTLPPSQEEMTKNQVSLTCLVKGFYPSDIAVEWESNGQPENNYKTTPPVLDSDGSFFLYSRLTVDKSRWQEGNVFSCSVMHEALHNHYTQKSLSLSLGK

SEQ ID NO: 38 - protein, 400 aa, synthetic construct
MMMDCDIEGKDGKQYESVLMVSIDQLLDSMKEIGSNCLNNEFNFFKRHICDANKEGMFLFRAARKLRQFLKMNSTGDFDLHLLKVSEGTTILLNCTGQVKGRKPAALGEAQPTKSLEENKSLKEQKKLNDLCFLKRLLQEIKTCWNKILMGTKEHRNTGRGGEEKKKEKEKEEQEERETKTPECPSHTQPLGVFLFPPKPKDTLMISRTPEVTCVVVDVSQEDPEVQFNWYVDGVEVHNAKTKPREEQFNSTYRVVSVLTVLHQDWLNGKEYKCKVSNKGLPSSIEKTISKAKGQPREPQVYTLPPSQEEMTKNQVSLTCLVKGFYPSDIAVEWESNGQPENNYKTTPPVLDSDGSFFLYSRLTVDKSRWQEGNVFSCSVMHEALHNHYTQKSLSLSLGK

SEQ ID NO: 39 - protein, 400 aa, synthetic construct
MGMDCDIEGKDGKQYESVLMVSIDQLLDSMKEIGSNCLNNEFNFFKRHICDANKEGMFLFRAARKLRQFLKMNSTGDFDLHLLKVSEGTTILLNCTGQVKGRKPAALGEAQPTKSLEENKSLKEQKKLNDLCFLKRLLQEIKTCWNKILMGTKEHRNTGRGGEEKKKEKEKEEQEERETKTPECPSHTQPLGVFLFPPKPKDTLMISRTPEVTCVVVDVSQEDPEVQFNWYVDGVEVHNAKTKPREEQFNSTYRVVSVLTVLHQDWLNGKEYKCKVSNKGLPSSIEKTISKAKGQPREPQVYTLPPSQEEMTKNQVSLTCLVKGFYPSDIAVEWESNGQPENNYKTTPPVLDSDGSFFLYSRLTVDKSRWQEGNVFSCSVMHEALHNHYTQKSLSLSLGK

SEQ ID NO: 40 - protein, 401 aa, synthetic construct
MMMMDCDIEGKDGKQYESVLMVSIDQLLDSMKEIGSNCLNNEFNFFKRHICDANKEGMFLFRAARKLRQFLKMNSTGDFDLHLLKVSEGTTILLNCTGQVKGRKPAALGEAQPTKSLEENKSLKEQKKLNDLCFLKRLLQEIKTCWNKILMGTKEHRNTGRGGEEKKKEKEKEEQEERETKTPECPSHTQPLGVFLFPPKPKDTLMISRTPEVTCVVVDVSQEDPEVQFNWYVDGVEVHNAKTKPREEQFNSTYRVVSVLTVLHQDWLNGKEYKCKVSNKGLPSSIEKTISKAKGQPREPQVYTLPPSQEEMTKNQVSLTCLVKGFYPSDIAVEWESNGQPENNYKTTPPVLDSDGSFFLYSRLTVDKSRWQEGNVFSCSVMHEALHNHYTQKSLSLSLGK

SEQ ID NO: 41 - protein, 397 aa, synthetic construct
DCDIEGKDGKQYESVLMVSIDQLLDSMKEIGSNCLNNEFNFFKRHICDANKEGMFLFRAARKLRQFLKMNSTGDFDLHLLKVSEGTTILLNCTGQVKGRKPAALGEAQPTKSLEENKSLKEQKKLNDLCFLKRLLQEIKTCWNKILMGTKEHRNTGRGGEEKKKEKEKEEQEERETKTPECPSHTQPLGVFLFPPKPKDTLMISRTPEVTCVVVDVSQEDPEVQFNWYVDGVEVHNAKTKPREEQFNSTYRVVSVLTVLHQDWLNGKEYKCKVSNKGLPSSIEKTISKAKGQPREPQVYTLPPSQEEMTKNQVSLTCLVKGFYPSDIAVEWESNGQPENNYKTTPPVLDSDGSFFLYSRLTVDKSRWQEGNVFSCSVMHEALHNHYTQKSLSLSLGK

SEQ ID NO: 42 - protein, 395 aa, synthetic construct
DCDIEGKDGKQYESVLMVSIDQLLDSMKEIGSNCLNNEFNFFKRHICDANKEGMFLFRAARKLRQFLKMNSTGDFDLHLLKVSEGTTILLNCTGQVKGRKPAALGEAQPTKSLEENKSLKEQKKLNDLCFLKRLLQEIKTCWNKILMGTKEHASAEPRGPTIKPCPPCKCPAPNLEGGPSVFIFPPKIKDVLMISLSPIVTCVVVDVSEDDPDVQISWFVNNVEVHTAQTQTHREDYNSTLRVVSALPIQHQDWMSGKAFACAVNNKDLPAPIERTISKPKGSVRAPQVYVLPPPEEEMTKKQVTLTCMVTDFMPEDIYVEWTNNGKTELNYKNTEPVLDSDGSYFMYSKLRVEKKNWVERNSYSCSVVHEGLHNHHTTKSFSRTPGKGGGNSGS

SEQ ID NO: 43 - DNA, 531 bp, Homo sapiens
  source 1..531: mol_type = genomic DNA
atgttccacgtgagcttcaggtacatcttcggcctgccacccctgatcctggtgctgctgcctgtggccagctccgactgcgacatcgagggaaaagacggcaagcagtacgaaagcgtgctgatggtgtccatcgaccagctgctggattctatgaaggagattgggagtaactgcctgaacaatgagttcaacttcttcaaacggcacatttgtgatgccaacaaggagggaatgttcctgtttcgggccgctagaaaactgaggcagttcctgaagatgaacagcaccggagactttgatctgcatctgctgaaagtgtctgagggcaccacaatcctgctgaactgcactgggcaggtgaaaggaaggaagcctgccgctctgggagaggctcagccaaccaagtcactggaggaaaacaaaagcctgaaggaacagaagaaactgaatgacctgtgctttctgaaacggctgctgcaggagatcaaaacatgttggaacaagattctgatgggcacaaaggaacac

SEQ ID NO: 44 - DNA, 534 bp, synthetic construct
  source 1..534: mol_type = other DNA
atgttccacgtgagcttcagatacatcttcggcctgccccccctgatcctggtgctgctgcccgtggccagcagcatggactgcgacatcgagggcaaggacggcaagcagtacgagagcgtgctgatggtgagcatcgaccagctgctggacagcatgaaggagatcggcagcaactgcctgaacaacgagttcaacttcttcaagagacacatctgcgacgccaacaaggagggcatgttcctgttcagagccgccagaaagctgagacagttcctgaagatgaacagcaccggcgacttcgacctgcacctgctgaaggtgagcgagggcacaaccatcctgctgaactgcaccggccaggtgaagggcagaaagcccgccgccctgggcgaggcccagcccaccaagagcctggaggagaacaagagcctgaaggagcagaagaagctgaacgacctgtgcttcctgaagagactgctgcaggagatcaagacctgctggaacaagatcctgatgggcaccaaggagcac

SEQ ID NO: 45 - DNA, 537 bp, synthetic construct
  source 1..537: mol_type = other DNA
atgttccacgtgagcttcagatacatcttcggcctgccccccctgatcctggtgctgctgcccgtggccagcagcatgatggactgcgacatcgagggcaaggacggcaagcagtacgagagcgtgctgatggtgagcatcgaccagctgctggacagcatgaaggagatcggcagcaactgcctgaacaacgagttcaacttcttcaagagacacatctgcgacgccaacaaggagggcatgttcctgttcagagccgccagaaagctgagacagttcctgaagatgaacagcaccggcgacttcgacctgcacctgctgaaggtgagcgagggcacaaccatcctgctgaactgcaccggccaggtgaagggcagaaagcccgccgccctgggcgaggcccagcccaccaagagcctggaggagaacaagagcctgaaggagcagaagaagctgaacgacctgtgcttcctgaagagactgctgcaggagatcaagacctgctggaacaagatcctgatgggcaccaaggagcac

SEQ ID NO: 46 - DNA, 540 bp, synthetic construct
  source 1..540: mol_type = other DNA
atgttccacgtgagcttcagatacatcttcggcctgccccccctgatcctggtgctgctgcccgtggccagcagcatgatgatggactgcgacatcgagggcaaggacggcaagcagtacgagagcgtgctgatggtgagcatcgaccagctgctggacagcatgaaggagatcggcagcaactgcctgaacaacgagttcaacttcttcaagagacacatctgcgacgccaacaaggagggcatgttcctgttcagagccgccagaaagctgagacagttcctgaagatgaacagcaccggcgacttcgacctgcacctgctgaaggtgagcgagggcacaaccatcctgctgaactgcaccggccaggtgaagggcagaaagcccgccgccctgggcgaggcccagcccaccaagagcctggaggagaacaagagcctgaaggagcagaagaagctgaacgacctgtgcttcctgaagagactgctgcaggagatcaagacctgctggaacaagatcctgatgggcaccaaggagcac

SEQ ID NO: 47 - DNA, 540 bp, synthetic construct
  source 1..540: mol_type = other DNA
atgttccacgtgagcttcaggtacatcttcggcctgccacccctgatcctggtgctgctgcctgtggccagctccatggggatggactgcgacatcgagggaaaagacggcaagcagtacgaaagcgtgctgatggtgtccatcgaccagctgctggattctatgaaggagattgggagtaactgcctgaacaatgagttcaacttcttcaaacggcacatttgtgatgccaacaaggagggaatgttcctgtttcgggccgctagaaaactgaggcagttcctgaagatgaacagcaccggagactttgatctgcatctgctgaaagtgtctgagggcaccacaatcctgctgaactgcactgggcaggtgaaaggaaggaagcctgccgctctgggagaggctcagccaaccaagtcactggaggaaaacaaaagcctgaaggaacagaagaaactgaatgacctgtgctttctgaaacggctgctgcaggagatcaaaacatgttggaacaagattctgatgggcaccaaggagcac

SEQ ID NO: 48 - DNA, 540 bp, synthetic construct
  source 1..540: mol_type = other DNA
atgttccacgtgagcttcagatacatcttcggcctgccccccctgatcctggtgctgctgcccgtggccagcagcgacgatgacgactgcgacatcgagggcaaggacggcaagcagtacgagagcgtgctgatggtgagcatcgaccagctgctggacagcatgaaggagatcggcagcaactgcctgaacaacgagttcaacttcttcaagagacacatctgcgacgccaacaaggagggcatgttcctgttcagagccgccagaaagctgagacagttcctgaagatgaacagcaccggcgacttcgacctgcacctgctgaaggtgagcgagggcacaaccatcctgctgaactgcaccggccaggtgaagggcagaaagcccgccgccctgggcgaggcccagcccaccaagagcctggaggagaacaagagcctgaaggagcagaagaagctgaacgacctgtgcttcctgaagagactgctgcaggagatcaagacctgctggaacaagatcctgatgggcaccaaggagcac

SEQ ID NO: 49 - DNA, 543 bp, synthetic construct
  source 1..543: mol_type = other DNA
atgttccacgtgagcttcagatacatcttcggcctgccccccctgatcctggtgctgctgcccgtggccagcagcatgatgatgatggactgcgacatcgagggcaaggacggcaagcagtacgagagcgtgctgatggtgagcatcgaccagctgctggacagcatgaaggagatcggcagcaactgcctgaacaacgagttcaacttcttcaagagacacatctgcgacgccaacaaggagggcatgttcctgttcagagccgccagaaagctgagacagttcctgaagatgaacagcaccggcgacttcgacctgcacctgctgaaggtgagcgagggcacaaccatcctgctgaactgcaccggccaggtgaagggcagaaagcccgccgccctgggcgaggcccagcccaccaagagcctggaggagaacaagagcctgaaggagcagaagaagctgaacgacctgtgcttcctgaagagactgctgcaggagatcaagacctgctggaacaagatcctgatgggcaccaaggagcac

SEQ ID NO: 50 - DNA, 1284 bp, synthetic construct
  source 1..1284: mol_type = other DNA
atgttccacgtgagcttcagatacatcttcggcctgccccccctgatcctggtgctgctgcccgtggccagcagcatggactgcgacatcgagggcaaggacggcaagcagtacgagagcgtgctgatggtgagcatcgaccagctgctggacagcatgaaggagatcggcagcaactgcctgaacaacgagttcaacttcttcaagagacacatctgcgacgccaacaaggagggcatgttcctgttcagagccgccagaaagctgagacagttcctgaagatgaacagcaccggcgacttcgacctgcacctgctgaaggtgagcgagggcacaaccatcctgctgaactgcaccggccaggtgaagggcagaaagcccgccgccctgggcgaggcccagcccaccaagagcctggaggagaacaagagcctgaaggagcagaagaagctgaacgacctgtgcttcctgaagagactgctgcaggagatcaagacctgctggaacaagatcctgatgggcaccaaggagcacaggaacacaggcagaggcggcgaggagaagaagaaggagaaggagaaggaggagcaggaggaaagagagaccaagacccccgagtgccccagccacacccagcccctgggcgtgttcctgttccctcccaagcccaaggacaccctgatgatcagcagaacccccgaggtgacctgcgtggtcgtggatgtgagccaggaagatcccgaagtgcagttcaactggtacgtggatggcgtggaagtgcacaacgccaagaccaagcccagagaagagcagttcaactccacctacagagtggtgagcgtgctgaccgtgctgcaccaggactggctgaacggcaaggagtacaagtgcaaggtgtccaacaaaggcctgcccagctccatcgagaagaccatcagcaaagccaaaggccagcccagagaaccccaggtgtacaccctgcctcccagccaggaagagatgaccaagaaccaggtgtccctgacctgcctggtgaaaggcttctaccccagcgacatcgccgtggagtgggaaagcaacggccagcccgagaacaattacaagacaacccctcccgtgctggatagcgatggcagcttctttctgtacagcagactgaccgtggacaagagcagatggcaggaaggcaacgtgttcagctgcagcgtgatgcacgaagccctgcacaaccactacacccagaagagcctgtccctgagcctgggcaagtgactcgagtctaga

SEQ ID NO: 51 - DNA, 1272 bp, synthetic construct
  source 1..1272: mol_type = other DNA
atgttccacgtgagcttcagatacatcttcggcctgccccccctgatcctggtgctgctgcccgtggccagcagcatgatggactgcgacatcgagggcaaggacggcaagcagtacgagagcgtgctgatggtgagcatcgaccagctgctggacagcatgaaggagatcggcagcaactgcctgaacaacgagttcaacttcttcaagagacacatctgcgacgccaacaaggagggcatgttcctgttcagagccgccagaaagctgagacagttcctgaagatgaacagcaccggcgacttcgacctgcacctgctgaaggtgagcgagggcacaaccatcctgctgaactgcaccggccaggtgaagggcagaaagcccgccgccctgggcgaggcccagcccaccaagagcctggaggagaacaagagcctgaaggagcagaagaagctgaacgacctgtgcttcctgaagagactgctgcaggagatcaagacctgctggaacaagatcctgatgggcaccaaggagcacaggaacacaggcagaggcggcgaggagaagaagaaggagaaggagaaggaggagcaggaggaaagagagaccaagacccccgagtgccccagccacacccagcccctgggcgtgttcctgttccctcccaagcccaaggacaccctgatgatcagcagaacccccgaggtgacctgcgtggtcgtggatgtgagccaggaagatcccgaagtgcagttcaactggtacgtggatggcgtggaagtgcacaacgccaagaccaagcccagagaagagcagttcaactccacctacagagtggtgagcgtgctgaccgtgctgcaccaggactggctgaacggcaaggagtacaagtgcaaggtgtccaacaaaggcctgcccagctccatcgagaagaccatcagcaaagccaaaggccagcccagagaaccccaggtgtacaccctgcctcccagccaggaagagatgaccaagaaccaggtgtccctgacctgcctggtgaaaggcttctaccccagcgacatcgccgtggagtgggaaagcaacggccagcccgagaacaattacaagacaacccctcccgtgctggatagcgatggcagcttctttctgtacagcagactgaccgtggacaagagcagatggcaggaaggcaacgtgttcagctgcagcgtgatgcacgaagccctgcacaaccactacacccagaagagcctgtccctgagcctgggcaag

SEQ ID NO: 52 - DNA, 1275 bp, synthetic construct
  source 1..1275: mol_type = other DNA
atgttccacgtgagcttcagatacatcttcggcctgccccccctgatcctggtgctgctgcccgtggccagcagcatgatgatggactgcgacatcgagggcaaggacggcaagcagtacgagagcgtgctgatggtgagcatcgaccagctgctggacagcatgaaggagatcggcagcaactgcctgaacaacgagttcaacttcttcaagagacacatctgcgacgccaacaaggagggcatgttcctgttcagagccgccagaaagctgagacagttcctgaagatgaacagcaccggcgacttcgacctgcacctgctgaaggtgagcgagggcacaaccatcctgctgaactgcaccggccaggtgaagggcagaaagcccgccgccctgggcgaggcccagcccaccaagagcctggaggagaacaagagcctgaaggagcagaagaagctgaacgacctgtgcttcctgaagagactgctgcaggagatcaagacctgctggaacaagatcctgatgggcaccaaggagcacaggaacacaggcagaggcggcgaggagaagaagaaggagaaggagaaggaggagcaggaggaaagagagaccaagacccccgagtgccccagccacacccagcccctgggcgtgttcctgttccctcccaagcccaaggacaccctgatgatcagcagaacccccgaggtgacctgcgtggtcgtggatgtgagccaggaagatcccgaagtgcagttcaactggtacgtggatggcgtggaagtgcacaacgccaagaccaagcccagagaagagcagttcaactccacctacagagtggtgagcgtgctgaccgtgctgcaccaggactggctgaacggcaaggagtacaagtgcaaggtgtccaacaaaggcctgcccagctccatcgagaagaccatcagcaaagccaaaggccagcccagagaaccccaggtgtacaccctgcctcccagccaggaagagatgaccaagaaccaggtgtccctgacctgcctggtgaaaggcttctaccccagcgacatcgccgtggagtgggaaagcaacggccagcccgagaacaattacaagacaacccctcccgtgctggatagcgatggcagcttctttctgtacagcagactgaccgtggacaagagcagatggcaggaaggcaacgtgttcagctgcagcgtgatgcacgaagccctgcacaaccactacacccagaagagcctgtccctgagcctgggcaag

SEQ ID NO: 53 - DNA, 1275 bp, synthetic construct
  source 1..1275: mol_type = other DNA
atgttccacgtgagcttcaggtacatcttcggcctgccacccctgatcctggtgctgctgcctgtggccagctccatggggatggactgcgacatcgagggaaaagacggcaagcagtacgaaagcgtgctgatggtgtccatcgaccagctgctggattctatgaaggagattgggagtaactgcctgaacaatgagttcaacttcttcaaacggcacatttgtgatgccaacaaggagggaatgttcctgtttcgggccgctagaaaactgaggcagttcctgaagatgaacagcaccggagactttgatctgcatctgctgaaagtgtctgagggcaccacaatcctgctgaactgcactgggcaggtgaaaggaaggaagcctgccgctctgggagaggctcagccaaccaagtcactggaggaaaacaaaagcctgaaggaacagaagaaactgaatgacctgtgctttctgaaacggctgctgcaggagatcaaaacatgttggaacaagattctgatgggcacaaaggaacaccgcaatactgggcggggcggggaggaaaagaaaaaggagaaggaaaaggaggaacaggaggaaagagagactaagaccccagaatgtcccagccatactcagcccctgggggtgttcctgtttccccctaaacctaaggataccctgatgatcagcaggacacccgaggtgacctgcgtggtcgtggatgtgagccaggaagatcccgaagtgcagttcaactggtacgtggatggcgtggaagtgcacaacgccaagaccaagcccagagaagagcagttcaactccacctacagagtggtgagcgtgctgaccgtgctgcaccaggactggctgaacggcaaggagtacaagtgcaaggtgtccaacaaaggcctgcccagctccatcgagaagaccatcagcaaagccaaaggccagcccagagaaccccaggtgtacaccctgcctcccagccaggaagagatgaccaagaaccaggtgtccctgacctgcctggtgaaaggcttctaccccagcgacatcgccgtggagtgggaaagcaacggccagcccgagaacaattacaagacaacccctcccgtgctggatagcgatggcagcttctttctgtacagcagactgaccgtggacaagagcagatggcaggaaggcaacgtgttcagctgcagcgtgatgcacgaagccctgcacaaccactacacccagaagagcctgtccctgagcctgggcaag

SEQ ID NO: 54 - DNA, 1278 bp, synthetic construct
  source 1..1278: mol_type = other DNA
atgttccacgtgagcttcagatacatcttcggcctgccccccctgatcctggtgctgctgcccgtggccagcagcatgatgatgatggactgcgacatcgagggcaaggacggcaagcagtacgagagcgtgctgatggtgagcatcgaccagctgctggacagcatgaaggagatcggcagcaactgcctgaacaacgagttcaacttcttcaagagacacatctgcgacgccaacaaggagggcatgttcctgttcagagccgccagaaagctgagacagttcctgaagatgaacagcaccggcgacttcgacctgcacctgctgaaggtgagcgagggcacaaccatcctgctgaactgcaccggccaggtgaagggcagaaagcccgccgccctgggcgaggcccagcccaccaagagcctggaggagaacaagagcctgaaggagcagaagaagctgaacgacctgtgcttcctgaagagactgctgcaggagatcaagacctgctggaacaagatcctgatgggcaccaaggagcacaggaacacaggcagaggcggcgaggagaagaagaaggagaaggagaaggaggagcaggaggaaagagagaccaagacccccgagtgccccagccacacccagcccctgggcgtgttcctgttccctcccaagcccaaggacaccctgatgatcagcagaacccccgaggtgacctgcgtggtcgtggatgtgagccaggaagatcccgaagtgcagttcaactggtacgtggatggcgtggaagtgcacaacgccaagaccaagcccagagaagagcagttcaactccacctacagagtggtgagcgtgctgaccgtgctgcaccaggactggctgaacggcaaggagtacaagtgcaaggtgtccaacaaaggcctgcccagctccatcgagaagaccatcagcaaagccaaaggccagcccagagaaccccaggtgtacaccctgcctcccagccaggaagagatgaccaagaaccaggtgtccctgacctgcctggtgaaaggcttctaccccagcgacatcgccgtggagtgggaaagcaacggccagcccgagaacaattacaagacaacccctcccgtgctggatagcgatggcagcttctttctgtacagcagactgaccgtggacaagagcagatggcaggaaggcaacgtgttcagctgcagcgtgatgcacgaagccctgcacaaccactacacccagaagagcctgtccctgagcctgggcaag

SEQ ID NO: 55 - protein, 4 aa, synthetic construct
MMMM